European Patent Application EP 4 201 961 A1, published June 28, 2023. Title: Antibody specifically bound to glycosylated CEACAM5. Applicant: Shanghai Genbase Biotechnology Co., LTD. The sequence listing filed with the application follows.

SEQUENCE LISTING (131 sequences)

SEQ ID NO: 1 - protein, 5 aa, Artificial Sequence
  M19 heavy chain variable region CDR1
DYFMN

SEQ ID NO: 2 - protein, 19 aa, Artificial Sequence
  M19 heavy chain variable region CDR2
QMRNKVNGDTTEYAESVEG

SEQ ID NO: 3 - protein, 10 aa, Artificial Sequence
  M19 heavy chain variable region CDR3
DKGIAYYFDY

SEQ ID NO: 4 - protein, 10 aa, Artificial Sequence
  M19 light chain variable region CDR1
RASSSVSYIH

SEQ ID NO: 5 - protein, 7 aa, Artificial Sequence
  M19 light chain variable region CDR2
GTSNLAS

SEQ ID NO: 6 - protein, 9 aa, Artificial Sequence
  M19 light chain variable region CDR3
QQWSSNLST

SEQ ID NO: 7 - protein, 5 aa, Artificial Sequence
  M7 heavy chain variable region CDR1
DDYMH

SEQ ID NO: 8 - protein, 17 aa, Artificial Sequence
  M7 heavy chain variable region CDR2
WIDPENGDTEYASKFQG

SEQ ID NO: 9 - protein, 13 aa, Artificial Sequence
  M7 heavy chain variable region CDR3
IYYVNPHYYAMDY

SEQ ID NO: 10 - protein, 10 aa, Artificial Sequence
  M7 light chain variable region CDR1
SATSSVSYMH

SEQ ID NO: 11 - protein, 7 aa, Artificial Sequence
  M7 light chain variable region CDR2
STSNLAS

SEQ ID NO: 12 - protein, 9 aa, Artificial Sequence
  M7 light chain variable region CDR3
QQRSSYPLT

SEQ ID NO: 13 - protein, 5 aa, Artificial Sequence
  M17 heavy chain variable region CDR1
DDYMH

SEQ ID NO: 14 - protein, 17 aa, Artificial Sequence
  M17 heavy chain variable region CDR2
WIDPENGDTEYASKFQG

SEQ ID NO: 15 - protein, 12 aa, Artificial Sequence
  M17 heavy chain variable region CDR3
IYYYGSRGAMDY

SEQ ID NO: 16 - protein, 10 aa, Artificial Sequence
  M17 light chain variable region CDR1
SASSSVSYMH

SEQ ID NO: 17 - protein, 7 aa, Artificial Sequence
  M17 light chain variable region CDR2
TTSTLAS

SEQ ID NO: 18 - protein, 9 aa, Artificial Sequence
  M17 light chain variable region CDR3
HQRSSYPLT

SEQ ID NO: 19 - protein, 5 aa, Artificial Sequence
  M18 heavy chain variable region CDR1
TYGMT

SEQ ID NO: 20 - protein, 17 aa, Artificial Sequence
  M18 heavy chain variable region CDR2
WINTYSGVPTYIDDFKG

SEQ ID NO: 21 - protein, 9 aa, Artificial Sequence
  M18 heavy chain variable region CDR3
KDLLGFMDY

SEQ ID NO: 22 - protein, 11 aa, Artificial Sequence
  M18 light chain variable region CDR1
KTSQDINKFMA

SEQ ID NO: 23 - protein, 7 aa, Artificial Sequence
  M18 light chain variable region CDR2
YTSTLQP

SEQ ID NO: 24 - protein, 9 aa, Artificial Sequence
  M18 light chain variable region CDR3
LQYDDLTWT

SEQ ID NO: 25 - protein, 140 aa, Artificial Sequence
  M19 heavy chain variable region
MGWSCIILFLVATATGVHSEVQLVESGGGLVQPGGSLRLSCAASGFTFTDYFMNWVRQAPGKALEWLGQMRNKVNGDTTEYAESVEGRFTISRDISKNSLYLQMNSLKTEDTAVYYCARDKGIAYYFDYWGQGTLVTVSS

SEQ ID NO: 26 - protein, 125 aa, Artificial Sequence
  M19 light chain variable region
MGWSCIILFLVATATGVHSDIQLTQSPSSLSASVGDRVTITCRASSSVSYIHWYQQKPGKSPKPWIHGTSNLASGVPSRFSGSGSGTDYTLTISSLQPEDAATYYCQQWSSNLSTFGQGTKLEIK

SEQ ID NO: 27 - protein, 122 aa, Artificial Sequence
  M7 heavy chain variable region
EVQLQQSGAELVRPGASVKLSCTVSGFNIKDDYMHWVKQRPEQGLEWIGWIDPENGDTEYASKFQGKATITADTSSNSAYLQLSSLTSEDTAVYYCTFIYYVNPHYYAMDYWGQGTSVTVSS

SEQ ID NO: 28 - protein, 106 aa, Artificial Sequence
  M7 light chain variable region
QIVLTQSPAIMSASPGEKVTITCSATSSVSYMHWFQQKPGTSPKLWIYSTSNLASGVPARFSGSGSGTSYSLTISRVEAEDAATYYCQQRSSYPLTFGAGTKLELK

SEQ ID NO: 29 - protein, 121 aa, Artificial Sequence
  M17 heavy chain variable region
EVQLQQSGAELVRPGASVKLSCTASGFNIKDDYMHWVKQRPEQGLEWIGWIDPENGDTEYASKFQGKATITADTSSNTAYLLLSSLTSEDTAVYYCTTIYYYGSRGAMDYWGQGTSVTVSS

SEQ ID NO: 30 - protein, 106 aa, Artificial Sequence
  M17 light chain variable region
QIVLTQSPAIMSASPGEKVTITCSASSSVSYMHWFQQKPGTSPKLWIYTTSTLASGVPARFSGSGSGTSYFLTISRMEAEDAATYYCHQRSSYPLTFGAGTKLELK

SEQ ID NO: 31 - protein, 118 aa, Artificial Sequence
  M18 heavy chain variable region
QIQLVQSGPELKKPGETVKISCKASGYTFTTYGMTWVKQAPGKGLKWMGWINTYSGVPTYIDDFKGRFAFSLETSASTAYLQINNLKNEDTATYFCGRKDLLGFMDYWGQGTSVTVSS

SEQ ID NO: 32 - protein, 106 aa, Artificial Sequence
  M18 light chain variable region
DIQMTQSPSSLSASLGGKVTITCKTSQDINKFMAWYQHKPGKGPRLLIRYTSTLQPGIPSRFSGSGSGRDYSFSIRNLEPEDIATYYCLQYDDLTWTFGGGTKLEI

SEQ ID NO: 33 - protein, 213 aa, Artificial Sequence
  antibody hMN14 light chain variable region
DIQLTQSPSSLSASVGDRVTITCKASQDVGTSVAWYQQKPGKAPKLLIYWTSTRHTGVPSRFSGSGSGTDFTFTISSLQPEDIATYYCQQYSLYRSFGQGTKVEIKRTVAAPSVFIFPPSDEQLKSGTASVVCLLNNFYPREAKVQWKVDNALQSGNSQESVTEQDSKDSTYSLSSTLTLSKADYEKHKVYACEVTHQGLSSPVTKSFNRGEC

SEQ ID NO: 34 - protein, 449 aa, Artificial Sequence
  antibody hMN14 heavy chain variable region
EVQLVESGGGVVQPGRSLRLSCSASGFDFTTYWMSWVRQAPGKGLEWIGEIHPDSSTINYAPSLKDRFTISRDNAKNTLFLQMDSLRPEDTGVYFCASLYFGFPWFAYWGQGTPVTVSSASTKGPSVFPLAPSSKSTSGGTAALGCLVKDYFPEPVTVSWNSGALTSGVHTFPAVLQSSGLYSLSSVVTVPSSSLGTQTYICNVNHKPSNTKVDKKVEPKSCDKTHTCPPCPAPELLGGPSVFLFPPKPKDTLMISRTPEVTCVVVDVSHEDPEVKFNWYVDGVEVHNAKTKPREEQYNSTYRVVSVLTVLHQDWLNGKEYKCKVSNKALPAPIEKTISKAKGQPREPQVYTLPPSREEMTKNQVSLTCLVKGFYPSDIAVEWESNGQPENNYKTTPPVLDSDGSFFLYSKLTVDKSRWQQGNVFSCSVMHEALHNHYTQKSLSLSPGK

SEQ ID NO: 35 - RNA, 12 nt, Artificial Sequence
  CEACAM5 KO1 sgRNA sequence
gacgacagacgg

SEQ ID NO: 36 - RNA, 16 nt, Artificial Sequence
  CEACAM5 KO2 sgRNA sequence
gagacgaacacgcgcc

SEQ ID NO: 37 - RNA, 16 nt, Artificial Sequence
  CEACAM5 KO3 sgRNA sequence
caggggagcaccacgg

SEQ ID NO: 38 - DNA, 417 bp, Artificial Sequence
  M19 heavy chain variable region nucleotide sequence
atgggctggagctgcatcatcctgttcctcgtggccacagctacaggagtgcatagcgaggtgcagctggtggaatcaggaggaggactggtgcagccaggaggatctctgagactgtcttgcgccgccagcggctttacattcaccgactacttcatgaattgggtccggcaggccccaggaaaagcactcgagtggctgggacagatgcggaacaaggtcaacggcgacaccacagagtacgccgaaagcgtggagggcagattcaccatcagccgggacatcagcaagaacagcctgtacctgcagatgaacagcctgaagaccgaggataccgccgtgtactattgcgccagggacaagggcatcgcctactacttcgactactggggccagggaacactggtgacagtgtct

SEQ ID NO: 39 - DNA, 375 bp, Artificial Sequence
  M19 light chain variable region nucleotide sequence
atgggctggagctgcatcatcctgttcctcgtggccacagctacaggagtgcatagcgacatccagctgacccagtctcctagcagcctgagcgccagcgtgggagatagagtgaccatcacttgcagagccagcagcagcgtgtcctacatccattggtaccagcagaagcccggcaagagccctaagccttggattcacggcaccagcaatctggccagcggagtgcctagcagattcagcggcagcggaagcggcaccgattacaccctgaccatcagctctctgcagccagaggacgcagccacctactattgccagcagtggagcagcaacctgagcacctttggccagggaaccaagctggagatcaag

SEQ ID NO: 40 - DNA, 366 bp, Artificial Sequence
  M7 heavy chain variable region nucleotide sequence
gaggttcagctgcagcagtctggggctgagcttgtgaggccaggggcctcagtcaagttgtcctgcacagtttctggctttaacattaaagacgactatatgcactgggtgaagcagaggcctgaacagggcctggagtggattggatggattgatcctgagaatggtgatactgaatatgcctcgaagttccagggcaaggccactataacagcagacacatcctccaactcagcctacctgcagctcagcagcctgacatctgaggacactgccgtctattactgtacttttatctactatgttaatcctcattactatgctatggactactggggtcaaggaacctcagtcaccgtctcctca

SEQ ID NO: 41 - DNA, 318 bp, Artificial Sequence
  M7 light chain variable region nucleotide sequence
caaattgttctcacccagtctccagcaatcatgtctgcttctccaggggagaaggtcaccatcacctgcagtgccacctcaagtgtaagttacatgcactggttccagcagaagccaggcacttctcccaaactctggatttatagcacatccaacctggcttctggagtccctgctcgcttcagtggcagtggatctgggacctcttactctctcacaatcagccgagtggaggctgaagatgctgccacttattactgccagcaaaggagtagttacccgctcacgttcggtgctgggaccaagctggagctgaaa

SEQ ID NO: 42 - DNA, 363 bp, Artificial Sequence
  M17 heavy chain variable region nucleotide sequence
gaggttcagctgcagcagtctggggctgagcttgtgaggccaggggcctcagtcaagttgtcctgcacagcttctggctttaacattaaagacgactatatgcactgggtgaagcagaggcctgaacagggcctggagtggattggatggattgatcctgagaatggtgatactgaatatgcctcgaagttccagggcaaggccactataacagcagacacatcctccaacacagcctacctgctgctcagcagcctgacatctgaggacactgccgtctattactgtactaccatttattactacggtagtagaggtgctatggactactggggtcaaggaacctcagtcaccgtctcctca

SEQ ID NO: 43 - DNA, 318 bp, Artificial Sequence
  M17 light chain variable region nucleotide sequence
caaattgttctcacccagtctccagcaatcatgtctgcatctccaggggagaaggtcaccataacctgcagtgccagctcaagtgtaagttacatgcactggttccagcagaagccaggcacttctcccaaactctggatttataccacatccaccctggcttctggagtccctgctcgcttcagtggcagtggatctgggacctcttactttctcacaatcagccgaatggaggctgaagatgctgccacttattactgccaccaaaggagtagttacccactcacgttcggtgctgggaccaagctggagctgaaa

SEQ ID NO: 44 - DNA, 354 bp, Artificial Sequence
  M18 heavy chain variable region nucleotide sequence
cagatccagttggtacagtctggacctgagctgaagaagcctggagagacagtcaagatctcctgcaaggcttctgggtatacctttacaacctatggaatgacctgggtgaaacaggctccaggaaagggtttaaagtggatgggctggataaacacctactctggagtgccaacatatattgatgacttcaagggacggtttgccttctctttggaaacctctgccagcactgcctatttgcagatcaacaacctcaaaaatgaggacacggctacatatttctgtggaagaaaggatctacttggttttatggactactggggtcaaggaacctcagtcaccgtctcctca

SEQ ID NO: 45 - DNA, 318 bp, Artificial Sequence
  M18 light chain variable region nucleotide sequence
gacatccagatgacacagtctccatcctcactgtctgcatctctgggaggcaaagtcaccatcacttgcaagacaagccaagacattaacaagtttatggcttggtaccaacacaagcctggaaaaggtcctaggctgctcatacgttacacatctacattacagccaggcatcccatcaaggttcagtggaagtgggtctgggagagattattccttcagcatcaggaacctggagcctgaagatattgcaacttattattgtctacagtatgatgatcttacgtggacgttcggtggaggcaccaagctggaaatc

SEQ ID NO: 46 - DNA, 940 bp, Artificial Sequence
  extracellular domain A1-B1-His nucleotide sequence
atgcacagctcagcactgctctgttgcctggtcctcctgactggggtgagggccaagctcactattgaatccacgccgttcaatgtcgcagaggggaaggaggtgcttctacttgtccacaatctgccccagcatctttttggctacagctggtacaaaggtgaaagagtggatggcaaccgtcaaattataggatatgtaataggaactcaacaagctaccccagggcccgcatacagtggtcgagagataatataccccaatgcatccctgctgatccagaacatcatccagaatgacacaggattctacaccctacacgtcataaagtcagatcttgtgaatgaagaagcaactggccagttccgggtatacccggagctgcccaagccctccatctccagcaacaactccaaacccgtggaggacaaggatgctgtggccttcacctgtgaacctgagactcaggacgcaacctacctgtggtgggtaaacaatcagagcctcccggtcagtcccaggctgcagctgtccaatggcaacaggaccctcactctattcaatgtcacaagaaatgacacagcaagctacaaatgtgaaacccagaacccagtgagtgccaggcgcagtgattcagtcatcctgaatgtcctctatggcccggatgcccccaccatttcccctctaaacacatcttacagatcaggggaaaatctgaacctctcctgccacgcagcctctaacccacctgcacagtactcttggtttgtcaatgggactttccagcaatccacccaagagctctttatccccaacatcactgtgaataatagtggatcctatacgtgccaagcccataactcagacactggcctcaataggaccacagtcacgacgatcacagtctatgcacaccatcaccatcaccattgagtctaga

SEQ ID NO: 47 - protein, 292 aa, Artificial Sequence
  extracellular domain A1-B1-His amino acid sequence
KLTIESTPFNVAEGKEVLLLVHNLPQHLFGYSWYKGERVDGNRQIIGYVIGTQQATPGPAYSGREIIYPNASLLIQNIIQNDTGFYTLHVIKSDLVNEEATGQFRVYPELPKPSISSNNSKPVEDKDAVAFTCEPETQDATYLWWVNNQSLPVSPRLQLSNGNRTLTLFNVTRNDTASYKCETQNPVSARRSDSVILNVLYGPDAPTISPLNTSYRSGENLNLSCHAASNPPAQYSWFVNGTFQQSTQELFIPNITVNNSGSYTCQAHNSDTGLNRTTVTTITVYAHHHHHH

SEQ ID NO: 48 - DNA, 616 bp, Artificial Sequence
  extracellular domain A2-B2-His nucleotide sequence
atgcacagctcagcactgctctgttgcctggtcctcctgactggggtgagggccgagccacccaaacccttcatcaccagcaacaactccaaccccgtggaggatgaggatgctgtagccttaacctgtgaacctgagattcagaacacaacctacctgtggtgggtaaataatcagagcctcccggtcagtcccaggctgcagctgtccaatgacaacaggaccctcactctactcagtgtcacaaggaatgatgtaggaccctatgagtgtggaatccagaacgaattaagtgttgaccacagcgacccagtcatcctgaatgtcctctatggcccagacgaccccaccatttccccctcatacacctattaccgtccaggggtgaacctcagcctctcctgccatgcagcctctaacccacctgcacagtattcttggctgattgatgggaacatccagcaacacacacaagagctctttatctccaacatcactgagaagaacagcggactctatacctgccaggccaataactcagccagtggccacagcaggactacagtcaagacaatcacagtctctgcgcaccatcaccatcaccattgagtctaga

SEQ ID NO: 49 - protein, 184 aa, Artificial Sequence
  extracellular domain A2-B2-His amino acid sequence
EPPKPFITSNNSNPVEDEDAVALTCEPEIQNTTYLWWVNNQSLPVSPRLQLSNDNRTLTLLSVTRNDVGPYECGIQNELSVDHSDPVILNVLYGPDDPTISPSYTYYRPGVNLSLSCHAASNPPAQYSWLIDGNIQQHTQELFISNITEKNSGLYTCQANNSASGHSRTTVKTITVSAHHHHHH

SEQ ID NO: 50 - DNA, 643 bp, Artificial Sequence
  extracellular domain A3-B3-His nucleotide sequence
atgcacagctcagcactgctctgttgcctggtcctcctgactggggtgagggccgagctgcccaagccctccatctccagcaacaactccaaacccgtggaggacaaggatgctgtggccttcacctgtgaacctgaggctcagaacacaacctacctgtggtgggtaaatggtcagagcctcccagtcagtcccaggctgcagctgtccaatggcaacaggaccctcactctattcaatgtcacaagaaatgacgcaagagcctatgtatgtggaatccagaactcagtgagtgcaaaccgcagtgacccagtcaccctggatgtcctctatgggccggacacccccatcatttcccccccagactcgtcttacctttcgggagcgaacctcaacctctcctgccactcggcctctaacccatccccgcagtattcttggcgtatcaatgggataccgcagcaacacacacaagttctctttatcgccaaaatcacgccaaataataacgggacctatgcctgttttgtctctaacttggctactggccgcaataattccatagtcaagagcatcacagtctctgcatctggaacttctcctggtctctcagctcaccatcaccatcaccattgagtctaga

SEQ ID NO: 51 - protein, 193 aa, Artificial Sequence [sequence omitted]

SEQ ID NO: 52 - DNA, 375 bp, Artificial Sequence
  humanized antibody hAb-009 light chain variable region nucleotide sequence
atgggctggagctgcatcatcctgttcctcgtggccacagctacaggagtgcatagcgagatcgtgctgacccagtctccagccacactgagcgcttctccaggagagagagccacactgtcttgtagagccagccagagcgtgtcctacatccattggtaccagcagaagcccggacagtctcctaggccttggattcacggcacaagcaatctggccaccggagtgccagctagattcagcggcagcggaagcggcaccgactttaccctgaccatcagctctctggagccagaggacgcagccgtgtactattgccagcagtggagcagcaatctgagcacctttggcggcggaaccaaggtggagatcaag

SEQ ID NO: 53 - DNA, 417 bp, Artificial Sequence
  humanized antibody hAb-009 heavy chain variable region nucleotide sequence
atgggctggagctgcatcatcctgttcctcgtggccacagctacaggagtgcatagcgaggtgcagctggtggaatcaggaggaggactggtgcagccaggaggatctctgagactgtcttgcgccgccagcggctttacattcaccgactactacatgaattgggtccggcaggccccaggaaaagcactcgagtggctgggcttcatccggaacaaggtcaacggcgacaccacagagtacgccgccagcgtgaagggcagattcaccatcagccgggacgacagcaagaacagcctgtacctgcagatgaacagcctgaagaccgaggataccgccgtgtactattgcgccagggacaagggcatcgcctactacttcgactactggggccagggaacactggtgacagtgtct

SEQ ID NO: 54 - DNA, 375 bp, Artificial Sequence
  humanized antibody hAb-003 light chain variable region nucleotide sequence
atgggctggagctgcatcatcctgttcctcgtggccacagctacaggagtgcatagcgacatccagatgacccagagccctagcagcctgagcgccagcgtgggagatagagtgaccatcacttgcagagccagcagcagcgtgtcctacatccattggtaccagcagaagcccggcaagagccctaagcccctgatctacggcaccagcaatctggccagcggagtgcctagcagattcagcggcagcggaagcggcaccgactttaccctgaccatcagctctctgcagccagaggacgcagccacctactattgccagcagtggagcagcaacctgagcacctttggccagggaaccaagctggagatcaag

SEQ ID NO: 55 - DNA, 417 bp, Artificial Sequence
  humanized antibody hAb-003 heavy chain variable region nucleotide sequence
atgggctggagctgcatcatcctgttcctcgtggccacagctacaggagtgcatagcgaggtgcagctggtggaatcaggaggaggactggtgcagccaggaggatctctgagactgtcttgcgccgccagcggctttacattcaccgactacttcatgaattgggtccggcaggccccaggaaaagcactcgagtgggtcggacagatgcggaacaaggtcaacggcgacaccacagagtacgccgagagcgtggagggaagattcaccatcagccgggacgacagcaagaacagcctgtacctgcagatgaacagcctgaagaccgaggataccgccgtgtactattgcgccagggacaagggcatcgcctactacttcgactactggggccagggaacactggtgacagtgtct

SEQ ID NO: 56 - DNA, 375 bp, Artificial Sequence
  humanized antibody hAb-005 light chain variable region nucleotide sequence
atgggctggagctgcatcatcctgttcctcgtggccacagctacaggagtgcatagcgacatccagctgacccagtctcctagcagcctgagcgccagcgtgggagatagagtgaccatcacttgcagagccagcagcagcgtgtcctacatccattggtaccagcagaagcccggcaagagccctaagccttggatctacggcaccagcaatctggccagcggagtgcctagcagattcagcggcagcggaagcggcaccgattacaccctgaccatcagctctctgcagccagaggacgcagccacctactattgccagcagtggagcagcaacctgagcacctttggccagggaaccaaggtggagatcaag

SEQ ID NO: 57 - DNA, 417 bp, Artificial Sequence
  humanized antibody hAb-005 heavy chain variable region nucleotide sequence
atgggctggagctgcatcatcctgttcctcgtggccacagctacaggagtgcatagcgaggtgcagctggtggaatcaggaggaggactggtgcagccaggaggatctctgagactgtcttgcgccgccagcggctttacattcaccgactacaccatgtcttgggtccggcaggcaccaggaaaagcactcgagtgggtcggcttcatccggaacaaggtcaacggcgacaccacagagtacagcgacagcgtggagggaaggttcaccatcagccgggacaacagcaagaacaccctgtacctgcagatgaacagcctgcgcgcagaggataccgccgtgtactattgcgccagggacaagggcatcgcctactacttcgactactggggccagggaacactggtgacagtgtct

SEQ ID NO: 58 - DNA, 375 bp, Artificial Sequence
  humanized antibody hAb-006 light chain variable region nucleotide sequence
atgggctggagctgcatcatcctgttcctcgtggccacagctacaggagtgcatagcgacatcgtgctgtctcagtctccaggcaccctgtctctgtctccaggagagagagccaccctgtcttgtagagccagcagcagcgtgtcctacatccattggtaccagcagaagcccggacaggctcctagaccttggattcacggcacaagcaatctggccagcggaatccccgacagattcagcggcagcggaagcggcaccgattacaccctgaccatcagcagactggagccagaggacttcgccgtgtactattgccagcagtggagcagcaatctgagcacctttggcggcggaaccaaggtggagatcaag

SEQ ID NO: 59 - DNA, 417 bp, Artificial Sequence
  humanized antibody hAb-006 heavy chain variable region nucleotide sequence
atgggctggagctgcatcatcctgttcctcgtggccacagctacaggagtgcatagcgaggtgcagctggtggaatcaggaggaggactggtgcagccaggaggatctctgagactgtcttgcgccgccagcggctttacattcaccgactactacatgaattgggtccggcaggccccaggaaaaggactcgagtggctgggcttcatccggaacaaggtcaacggcgacaccaccgagtacagcgccagcgtgaagggcaggttcaccatcagccgggacatcagcaagaacagcctgtacctgcagatgaacagcctgaagaccgaggataccgccgtgtactattgcgccagggacaagggcatcgcctactacttcgactactggggccagggaacactggtgacagtgtct

SEQ ID NO: 60 - DNA, 375 bp, Artificial Sequence
  humanized antibody hAb-010 light chain variable region nucleotide sequence
atgggctggagctgcatcatcctgttcctcgtggccacagctacaggagtgcatagcgagatcgtgctgacccagtctccagccacactgagcgcttctccaggagagagagccacactgtcttgcagagccagctctagcgtgtcctacatccattggtaccagcagaagcccggccagtctcctagacccctgatctacggcaccagcaacagagccacaggcgtgccagctagattcagcggcagcggaagcggcaccgactttaccctgaccatcagctctctggagccagaggacgcagccgtgtactattgccagcagtggagcagcaatctgagcacctttggcggcggaaccaaggtggagatcaag

SEQ ID NO: 61 - DNA, 417 bp, Artificial Sequence
  humanized antibody hAb-010 heavy chain variable region nucleotide sequence
atgggctggagctgcatcatcctgttcctcgtggccacagctacaggagtgcatagcgaggtgcagctggtggaatcaggaggaggactggtgcagccaggaggatctctgagactgtcttgcgccgccagcggctttacattcaccgactactacatggattgggtccggcaggctccaggaaaagcactcgagtgggtcggcttcatccggaacaaggtcaacggcgacaccacagagtacgccgccagcgtgaagggcagattcaccatcagccgggacgacagcaagaacagcctgtacctgcagatgaacagcctgaagaccgaggataccgccgtgtactattgcgccagggacaagggcatcgcctactacttcgactactggggccagggaacactggtgacagtgtct

SEQ ID NO: 62 - DNA, 375 bp, Artificial Sequence
  humanized antibody hAb-013 light chain variable region nucleotide sequence
atgggctggagctgcatcatcctgttcctcgtggccacagctacaggagtgcatagccagatcgtgctgacccagtctccagccacactgagcgcttctccaggagagagagccacactgtcttgcagagccagctctagcgtgtcctacatccattggtaccagcagaagcccggacagagccctagacctctgatctacggcaccagcaatctggccagcggagtgccagctagattcagcggcagcggaagcggcaccgactttaccctgaccatcagctctctggagccagaggacgcagccgtgtactattgccagcagtggagcagcaatctgagcacctttggcggcggaaccaaggtggagatcaag

SEQ ID NO: 63 - DNA, 417 bp, Artificial Sequence
  humanized antibody hAb-013 heavy chain variable region nucleotide sequence
atgggctggagctgcatcatcctgttcctcgtggccacagctacaggagtgcatagcgaggtgcagctggtggaatcaggaggaggactggtgcagccaggaggatctctgagactgtcttgcgccgccagcggctttacattcaccgactactacatggattgggtccggcaggctccaggaaaagcactcgagtgggtcggcttcacccggaacaaggtcaacggcgacaccacagagtacgccgccagcgtgaagggcagattcaccatcagccgggacgacagcaagaacagcctgtacctgcagatgaacagcctgaagaccgaggataccgccgtgtactattgcgccagggacaagggcatcgcctactacttcgactactggggccagggaacactggtgacagtgtct

SEQ ID NO: 64 - DNA, 375 bp, Artificial Sequence
  humanized antibody hAb-016 light chain variable region nucleotide sequence
atgggctggagctgcatcatcctgttcctcgtggccacagctacaggagtgcatagcgagatcgtgctgacccagtctccaggcacactgagcgcttctccaggagagagagccacactgtcttgcagagccagctctagcgtgtcctacatccattggtaccagcagaagcccggacagagccctagacctctgatctacggcaccagcaatctggccagcggagtgccagacagattcagcggcagcggaagcggcaccgactttaccctgaccatcagcagactggagccagaggacgcagccgtgtactattgccagcagtggagcagcaatctgagcacctttggcggcggaaccaaggtggagatcaag

SEQ ID NO: 65 - DNA, 417 bp, Artificial Sequence; identical to SEQ ID NO: 63
  humanized antibody hAb-016 heavy chain variable region nucleotide sequence

SEQ ID NO: 66 - DNA, 375 bp, Artificial Sequence
  humanized antibody hAb-017 light chain variable region nucleotide sequence
atgggctggagctgcatcatcctgttcctcgtggccacagctacaggagtgcatagcgagatcgtgctgacccagtctccagccacactgagcgcttctccaggagagagagccacactgtcttgcagagccagctctagcgtgtcctacatccattggtaccagcagaagcccggccagtctcctagacctctgatctacggcgccagcaatctggccagcggcgtgccagccagattcagcggaagcggcagcggcaccgactttaccctgaccatcagctctctggagccagaggacgcagccgtgtactattgccagcagtggagcagcaatctgagcacctttggcggcggaaccaaggtggagatcaag

SEQ ID NO: 67 - DNA, 417 bp, Artificial Sequence; identical to SEQ ID NO: 63
  humanized antibody hAb-017 heavy chain variable region nucleotide sequence

SEQ ID NO: 68 - protein, 125 aa, Artificial Sequence
  humanized antibody hAb-009 light chain variable region amino acid sequence
MGWSCIILFLVATATGVHSEIVLTQSPATLSASPGERATLSCRASQSVSYIHWYQQKPGQSPRPWIHGTSNLATGVPARFSGSGSGTDFTLTISSLEPEDAAVYYCQQWSSNLSTFGGGTKVEIK

SEQ ID NO: 69 - protein, 140 aa, Artificial Sequence
  humanized antibody hAb-009 heavy chain variable region amino acid sequence
MGWSCIILFLVATATGVHSEVQLVESGGGLVQPGGSLRLSCAASGFTFTDYYMNWVRQAPGKALEWLGFIRNKVNGDTTEYAASVKGRFTISRDDSKNSLYLQMNSLKTEDTAVYYCARDKGIAYYFDYWGQGTLVTVSS

SEQ ID NO: 70 - protein, 125 aa, Artificial Sequence
  humanized antibody hAb-003 light chain variable region amino acid sequence
MGWSCIILFLVATATGVHSDIQMTQSPSSLSASVGDRVTITCRASSSVSYIHWYQQKPGKSPKPLIYGTSNLASGVPSRFSGSGSGTDFTLTISSLQPEDAATYYCQQWSSNLSTFGQGTKLEIK

SEQ ID NO: 71 - protein, 140 aa, Artificial Sequence
  humanized antibody hAb-003 heavy chain variable region amino acid sequence
MGWSCIILFLVATATGVHSEVQLVESGGGLVQPGGSLRLSCAASGFTFTDYFMNWVRQAPGKALEWVGQMRNKVNGDTTEYAESVEGRFTISRDDSKNSLYLQMNSLKTEDTAVYYCARDKGIAYYFDYWGQGTLVTVSS

SEQ ID NO: 72 - protein, 125 aa, Artificial Sequence
  humanized antibody hAb-005 light chain variable region amino acid sequence
MGWSCIILFLVATATGVHSDIQLTQSPSSLSASVGDRVTITCRASSSVSYIHWYQQKPGKSPKPWIYGTSNLASGVPSRFSGSGSGTDYTLTISSLQPEDAATYYCQQWSSNLSTFGQGTKVEIK

SEQ ID NO: 73 - protein, 140 aa, Artificial Sequence
  humanized antibody hAb-005 heavy chain variable region amino acid sequence
MGWSCIILFLVATATGVHSEVQLVESGGGLVQPGGSLRLSCAASGFTFTDYTMSWVRQAPGKALEWVGFIRNKVNGDTTEYSDSVEGRFTISRDNSKNTLYLQMNSLRAEDTAVYYCARDKGIAYYFDYWGQGTLVTVSS

SEQ ID NO: 74 - protein, 125 aa, Artificial Sequence
  humanized antibody hAb-006 light chain variable region amino acid sequence
MGWSCIILFLVATATGVHSDIVLSQSPGTLSLSPGERATLSCRASSSVSYIHWYQQKPGQAPRPWIHGTSNLASGIPDRFSGSGSGTDYTLTISRLEPEDFAVYYCQQWSSNLSTFGGGTKVEIK

SEQ ID NO: 75 - protein, 140 aa, Artificial Sequence
  humanized antibody hAb-006 heavy chain variable region amino acid sequence
MGWSCIILFLVATATGVHSEVQLVESGGGLVQPGGSLRLSCAASGFTFTDYYMNWVRQAPGKGLEWLGFIRNKVNGDTTEYSASVKGRFTISRDISKNSLYLQMNSLKTEDTAVYYCARDKGIAYYFDYWGQGTLVTVSS

SEQ ID NO: 76 - protein, 125 aa, Artificial Sequence
  humanized antibody hAb-010 light chain variable region amino acid sequence
MGWSCIILFLVATATGVHSEIVLTQSPATLSASPGERATLSCRASSSVSYIHWYQQKPGQSPRPLIYGTSNRATGVPARFSGSGSGTDFTLTISSLEPEDAAVYYCQQWSSNLSTFGGGTKVEIK

SEQ ID NO: 77 - protein, 140 aa, Artificial Sequence
  humanized antibody hAb-010 heavy chain variable region amino acid sequence
MGWSCIILFLVATATGVHSEVQLVESGGGLVQPGGSLRLSCAASGFTFTDYYMDWVRQAPGKALEWVGFIRNKVNGDTTEYAASVKGRFTISRDDSKNSLYLQMNSLKTEDTAVYYCARDKGIAYYFDYWGQGTLVTVSS

SEQ ID NO: 78 - protein, 125 aa, Artificial Sequence
  humanized antibody hAb-013 light chain variable region amino acid sequence
MGWSCIILFLVATATGVHSQIVLTQSPATLSASPGERATLSCRASSSVSYIHWYQQKPGQSPRPLIYGTSNLASGVPARFSGSGSGTDFTLTISSLEPEDAAVYYCQQWSSNLSTFGGGTKVEIK

SEQ ID NO: 79 - protein, 140 aa, Artificial Sequence
  humanized antibody hAb-013 heavy chain variable region amino acid sequence
MGWSCIILFLVATATGVHSEVQLVESGGGLVQPGGSLRLSCAASGFTFTDYYMDWVRQAPGKALEWVGFTRNKVNGDTTEYAASVKGRFTISRDDSKNSLYLQMNSLKTEDTAVYYCARDKGIAYYFDYWGQGTLVTVSS

SEQ ID NO: 80 - protein, 125 aa, Artificial Sequence
  humanized antibody hAb-016 light chain variable region amino acid sequence
MGWSCIILFLVATATGVHSEIVLTQSPGTLSASPGERATLSCRASSSVSYIHWYQQKPGQSPRPLIYGTSNLASGVPDRFSGSGSGTDFTLTISRLEPEDAAVYYCQQWSSNLSTFGGGTKVEIK

SEQ ID NO: 81 - protein, 140 aa, Artificial Sequence; identical to SEQ ID NO: 79
  humanized antibody hAb-016 heavy chain variable region amino acid sequence

SEQ ID NO: 82 - protein, 125 aa, Artificial Sequence
  humanized antibody hAb-017 light chain variable region amino acid sequence
MGWSCIILFLVATATGVHSEIVLTQSPATLSASPGERATLSCRASSSVSYIHWYQQKPGQSPRPLIYGASNLASGVPARFSGSGSGTDFTLTISSLEPEDAAVYYCQQWSSNLSTFGGGTKVEIK

SEQ ID NO: 83 - protein, 140 aa, Artificial Sequence; identical to SEQ ID NO: 79
  humanized antibody hAb-017 heavy chain variable region amino acid sequence

SEQ ID NO: 84 - protein, 10 aa, Artificial Sequence
  humanized antibody hAb-009 light chain variable region CDR1 sequence
RASQSVSYIH

SEQ ID NO: 85 - protein, 7 aa, Artificial Sequence
  humanized antibody hAb-009 light chain variable region CDR2 sequence
GTSNLAT

SEQ ID NO: 86 - protein, 9 aa, Artificial Sequence
  humanized antibody hAb-009 light chain variable region CDR3 sequence
QQWSSNLST

SEQ ID NO: 87 - protein, 5 aa, Artificial Sequence
  humanized antibody hAb-009 heavy chain variable region CDR1 sequence
DYYMN

SEQ ID NO: 88 - protein, 19 aa, Artificial Sequence
  humanized antibody hAb-009 heavy chain variable region CDR2 sequence
FIRNKVNGDTTEYAASVKG

SEQ ID NO: 89 - protein, 10 aa, Artificial Sequence
  humanized antibody hAb-009 heavy chain variable region CDR3 sequence
DKGIAYYFDY

SEQ ID NO: 90 - protein, 10 aa, Artificial Sequence
  humanized antibody hAb-003 light chain variable region CDR1 sequence
RASSSVSYIH

SEQ ID NO: 91 - protein, 7 aa, Artificial Sequence
  humanized antibody hAb-003 light chain variable region CDR2 sequence
GTSNLAS

SEQ ID NO: 92 - protein, 9 aa, Artificial Sequence
  humanized antibody hAb-003 light chain variable region CDR3 sequence
QQWSSNLST

SEQ ID NO: 93 - protein, 5 aa, Artificial Sequence
  humanized antibody hAb-003 heavy chain variable region CDR1 sequence
DYFMN

SEQ ID NO: 94 - protein, 19 aa, Artificial Sequence
  humanized antibody hAb-003 heavy chain variable region CDR2 sequence
QMRNKVNGDTTEYAESVEG

SEQ ID NO: 95 - protein, 10 aa, Artificial Sequence
  humanized antibody hAb-003 heavy chain variable region CDR3 sequence
DKGIAYYFDY

SEQ ID NO: 96 - protein, 10 aa, Artificial Sequence
  humanized antibody hAb-005 light chain variable region CDR1 sequence
RASSSVSYIH

SEQ ID NO: 97 - protein, 7 aa, Artificial Sequence
  humanized antibody hAb-005 light chain variable region CDR2 sequence
GTSNLAS

SEQ ID NO: 98 - protein, 9 aa, Artificial Sequence
  humanized antibody hAb-005 light chain variable region CDR3 sequence
QQWSSNLST

SEQ ID NO: 99 - protein, 5 aa, Artificial Sequence
  humanized antibody hAb-005 heavy chain variable region CDR1 sequence
DYTMS

SEQ ID NO: 100 - protein, 19 aa, Artificial Sequence
  humanized antibody hAb-005 heavy chain variable region CDR2 sequence
FIRNKVNGDTTEYSDSVEG

SEQ ID NO: 101 - protein, 10 aa, Artificial Sequence
  humanized antibody hAb-005 heavy chain variable region CDR3 sequence
DKGIAYYFDY

SEQ ID NO: 102 - protein, 10 aa, Artificial Sequence
  humanized antibody hAb-006 light chain variable region CDR1 sequence
RASSSVSYIH

SEQ ID NO: 103 - protein, 7 aa, Artificial Sequence
  humanized antibody hAb-006 light chain variable region CDR2 sequence
GTSNLAS

SEQ ID NO: 104 - protein, 9 aa, Artificial Sequence
  humanized antibody hAb-006 light chain variable region CDR3 sequence
QQWSSNLST

SEQ ID NO: 105 - protein, 5 aa, Artificial Sequence
  humanized antibody hAb-006 heavy chain variable region CDR1 sequence
DYYMN

SEQ ID NO: 106 - protein, 19 aa, Artificial Sequence
  humanized antibody hAb-006 heavy chain variable region CDR2 sequence
FIRNKVNGDTTEYSASVKG

SEQ ID NO: 107 - protein, 10 aa, Artificial Sequence
  humanized antibody hAb-006 heavy chain variable region CDR3 sequence
DKGIAYYFDY

SEQ ID NO: 108 - protein, 10 aa, Artificial Sequence
  humanized antibody hAb-010 light chain variable region CDR1 sequence
RASSSVSYIH

SEQ ID NO: 109 - protein, 7 aa, Artificial Sequence
  humanized antibody hAb-010 light chain variable region CDR2 sequence
GTSNRAT

SEQ ID NO: 110 - protein, 9 aa, Artificial Sequence
  humanized antibody hAb-010 light chain variable region CDR3 sequence
QQWSSNLST

SEQ ID NO: 111 - protein, 5 aa, Artificial Sequence
  humanized antibody hAb-010 heavy chain variable region CDR1 sequence
DYYMD

SEQ ID NO: 112 - protein, 19 aa, Artificial Sequence
  humanized antibody hAb-010 heavy chain variable region CDR2 sequence
FIRNKVNGDTTEYAASVKG

SEQ ID NO: 113 - protein, 10 aa, Artificial Sequence
  humanized antibody hAb-010 heavy chain variable region CDR3 sequence
DKGIAYYFDY

SEQ ID NO: 114 - protein, 10 aa, Artificial Sequence
  humanized antibody hAb-013 light chain variable region CDR1 sequence
RASSSVSYIH

SEQ ID NO: 115 - protein, 7 aa, Artificial Sequence
  humanized antibody hAb-013 light chain variable region CDR2 sequence
GTSNLAS

SEQ ID NO: 116 - protein, 9 aa, Artificial Sequence
  humanized antibody hAb-013 light chain variable region CDR3 sequence
QQWSSNLST

SEQ ID NO: 117 - protein, 5 aa, Artificial Sequence
  humanized antibody hAb-013 heavy chain variable region CDR1 sequence
DYYMD

SEQ ID NO: 118 - protein, 19 aa, Artificial Sequence
  humanized antibody hAb-013 heavy chain variable region CDR2 sequence
FTRNKVNGDTTEYAASVKG

SEQ ID NO: 119 - protein, 10 aa, Artificial Sequence
  humanized antibody hAb-013 heavy chain variable region CDR3 sequence
DKGIAYYFDY

SEQ ID NO: 120 - protein, 10 aa, Artificial Sequence
  humanized antibody hAb-016 light chain variable region CDR1 sequence
RASSSVSYIH

SEQ ID NO: 121 - protein, 7 aa, Artificial Sequence
  humanized antibody hAb-016 light chain variable region CDR2 sequence
GTSNLAS

SEQ ID NO: 122 - protein, 9 aa, Artificial Sequence
  humanized antibody hAb-016 light chain variable region CDR3 sequence
QQWSSNLST

SEQ ID NO: 123 - protein, 5 aa, Artificial Sequence
  humanized antibody hAb-016 heavy chain variable region CDR1 sequence
DYYMD

SEQ ID NO: 124 - protein, 19 aa, Artificial Sequence
  humanized antibody hAb-016 heavy chain variable region CDR2 sequence
FTRNKVNGDTTEYAASVKG

SEQ ID NO: 125 - protein, 10 aa, Artificial Sequence
  humanized antibody hAb-016 heavy chain variable region CDR3 sequence
DKGIAYYFDY

SEQ ID NO: 126 - protein, 10 aa, Artificial Sequence
  humanized antibody hAb-017 light chain variable region CDR1 sequence
RASSSVSYIH

SEQ ID NO: 127 - protein, 7 aa, Artificial Sequence
  humanized antibody hAb-017 light chain variable region CDR2 sequence
GASNLAS

SEQ ID NO: 128 - protein, 9 aa, Artificial Sequence
  humanized antibody hAb-017 light chain variable region CDR3 sequence
QQWSSNLST

SEQ ID NO: 129 - protein, 5 aa, Artificial Sequence
  humanized antibody hAb-017 heavy chain variable region CDR1 sequence
DYYMD

SEQ ID NO: 130 - protein, 19 aa, Artificial Sequence
  humanized antibody hAb-017 heavy chain variable region CDR2 sequence
FTRNKVNGDTTEYAASVKG

SEQ ID NO: 131 - protein, 10 aa, Artificial Sequence
  humanized antibody hAb-017 heavy chain variable region CDR3 sequence
DKGIAYYFDY